European Patent Specification EP 4 263 586 B1, published March 11, 2026. Title: POLYPEPTIDES AND USES THEREOF. Applicant: MEDIMMUNE LIMITED. The sequence listing filed with the application follows.

SEQUENCE LISTING (159 sequences)

SEQ ID NO: 1 - protein, 37 aa, Artificial Sequence
  source: /note="Description of Artificial Sequence: Synthetic polypeptide"
  SITE (2)..(7): /note"Disulphide bridge between Cys residues"
KCNTATCATQRLANFLVHSSNNFGPILPPTNVGSNTY

SEQ ID NO: 2 - protein, 41 aa, Artificial Sequence
  source: /note="Description of Artificial Sequence: Synthetic polypeptide"
  MOD_RES (1)..(1): Lys (albumin binding moiety) or absent
  VARIANT (2)..(2): /replace=" "
  VARIANT (3)..(3): /replace=" "
  VARIANT (4)..(4): /replace="Lys (albumin binding moiety)" or " "
  VARIANT (5)..(5): /replace="Lys (albumin binding moiety)" or " "
  VARIANT (8)..(8): /replace="Ile" or "Ala"
  VARIANT (18)..(18): /replace="His" or "Glu" or "2,4-diaminobutanoic acid (Dab)" or "alpha methyl amino acid"
  VARIANT (19)..(19): /replace="Trp"
  VARIANT (20)..(20): /replace="D-Leu"
  VARIANT (21)..(21): /replace="Ser" or "Glu" or "Arg" or "(2S,4R)-4-hydroxypyrrolidine -2-carboxylic acid (Hyp)" or "Dab" or "alpha methyl amino acid"
  VARIANT (24)..(24): /replace="Ile" or "Pro" or "alpha methyl amino acid"
  VARIANT (25)..(25): /replace="Dab" or "His" or "Pro" or "Ser" or "Arg" or "Lys" or "Gly" or "Glu" or "Ala" or "Hyp " or "alpha methyl amino acid"
  VARIANT (26)..(26): /replace="His" or "Hyp" or "Dab" or "alpha methyl amino acid"
  VARIANT (27)..(27): /replace="Hyp" or "alpha methyl amino acid"
  VARIANT (28)..(28): /replace="Pro" or "Hyp" or "alpha methyl amino acid"
  VARIANT (29)..(29): /replace="Ala" or "Hyp" or "alpha methyl amino acid"
  VARIANT (30)..(30): /replace="D-Ile" or "Arg" or "Hyp" or "alpha methyl amino acid"
  VARIANT (31)..(31): /replace="D-Leu" or "Hyp" or "alpha methyl amino acid"
  VARIANT (32)..(32): /replace="D-Pro" or "Ser" or "Hyp" or "alpha methyl amino acid"
  VARIANT (33)..(33): /replace="Hyp" or "alpha methyl amino acid"
  VARIANT (35)..(35): /replace="Glu" or "His" or "Arg" or "Pro" or "Dab" or "alpha methyl amino acid"
  VARIANT (36)..(36): /replace="Hyp" or "Dab" or "alpha methyl amino acid"
  VARIANT (37)..(37): /replace="Pro" or "Hyp" or "alpha methyl amino acid"
  VARIANT (38)..(38): /replace="Pro" or "His" or "Hyp" or "alpha methyl amino acid"
  VARIANT (39)..(39): /replace="Pro" or "Arg" or "Glu" or "Dab" or "Hyp" or "alpha methyl amino acid"
  VARIANT (40)..(40): /replace="Hyp" or "alpha methyl amino acid"
  VARIANT (41)..(41): /replace="Pro" or "Hyp" or "alpha methyl amino acid"
  SITE (1)..(41): /note="Variant residues given in the sequence have no preference with respect to those in the annotations for variant positions"
XGGGKCNTATCATQRLANFLVHSSNNFGPILPPTNVGSNTY

SEQ ID NO: 3 - protein, 38 aa, Artificial Sequence
  source: /note="Description of Artificial Sequence: Synthetic polypeptide"
  MOD_RES (1)..(1): C18diacid-gamma-Glu
  SITE (3)..(8): /note"Disulphide bridge between Cys residues"
XKCNTATCATQRLANFLVHSSNNFGPILPPTNVGSNTY

SEQ ID NO: 4 - protein, 42 aa, Artificial Sequence
  source: /note="Description of Artificial Sequence: Synthetic polypeptide"
  MOD_RES (1)..(1): C18diacid-gamma-Glu
  MOD_RES (2)..(2): gamma-Glu
  SITE (7)..(12): /note"Disulphide bridge between Cys residues"
XXGGGKCNTATCATQRLANFLVHSSNNFGPILPPTNVGSNTY

SEQ ID NO: 5 - protein, 37 aa, Artificial Sequence
  source: /note="Description of Artificial Sequence: Synthetic polypeptide"
  MOD_RES (1)..(1): Lys, wherein the side chain of Lys is connected to gamma-Glu-gamma-Glu-C18diacid
  SITE (2)..(7): /note"Disulphide bridge between Cys residues"
XCNTATCATQRLANFLVHSSNNFGPILPPTNVGSNTY

SEQ ID NO: 6 - protein, 37 aa, Artificial Sequence; identical to SEQ ID NO: 5
  source: /note="Description of Artificial Sequence: Synthetic polypeptide"
  MOD_RES (1)..(1): Lys, wherein the side chain of Lys is connected to O2Oc-O2Oc-gamma-Glu-C18diacid
  SITE (2)..(7): /note"Disulphide bridge between Cys residues"

SEQ ID NO: 7 - protein, 41 aa, Artificial Sequence; identical to SEQ ID NO: 2
  source: /note="Description of Artificial Sequence: Synthetic polypeptide"
  MOD_RES (1)..(1): Lys, wherein the side chain of Lys is connected to O2Oc-O2Oc-gamma-Glu-C18diacid
  SITE (6)..(11): /note"Disulphide bridge between Cys residues"

SEQ ID NO: 8 - protein, 37 aa, Artificial Sequence
  source: /note="Description of Artificial Sequence: Synthetic polypeptide"
  MOD_RES (1)..(1): Lys, wherein the side chain of Lys is connected to gamma-Glu-gamma-Glu-C18diacid
  SITE (2)..(7): /note"Disulphide bridge between Cys residues"
  MOD_RES (21)..(21): 2,4-diaminobutanoic acid
XCNTATCATQRLANFLVHSSXNFPAILSPTNVGSNTY

SEQ ID NO: 9 - protein, 37 aa, Artificial Sequence; identical to SEQ ID NO: 8
  source: /note="Description of Artificial Sequence: Synthetic polypeptide"
  MOD_RES (1)..(1): Lys, wherein the side chain of Lys is connected to gamma-Glu-gamma-Glu-C18diacid
  SITE (2)..(7): /note"Disulphide bridge between Cys residues"
  MOD_RES (21)..(21): 2-amino-2-methylpropanoic acid

SEQ ID NO: 10 - protein, 37 aa, Artificial Sequence
  source: /note="Description of Artificial Sequence: Synthetic polypeptide"
  MOD_RES (1)..(1): C18diacid-gamma-Glu
  SITE (2)..(7): /note"Disulphide bridge between Cys residues"
  MOD_RES (23)..(23): (S)-2-amino-2-methyl-3-phenylpropanoic acid
XCNTATCATQRLAEFLRHSSNNXGPILPPTNVGSNTY

SEQ ID NO: 11 - protein, 37 aa, Artificial Sequence; identical to SEQ ID NO: 10
  source: /note="Description of Artificial Sequence: Synthetic polypeptide"
  MOD_RES (1)..(1): Lys, wherein the side chain of Lys is connected to gamma-Glu-gamma-Glu-C18diacid
  SITE (2)..(7): /note"Disulphide bridge between Cys residues"
  MOD_RES (23)..(23): (S)-2-amino-2-methyl-3-phenylpropanoic acid

SEQ ID NO: 12 - protein, 38 aa, Artificial Sequence
  source: /note="Description of Artificial Sequence: Synthetic polypeptide"
  MOD_RES (1)..(1): Lys, wherein the side chain of Lys is connected to gamma-Glu-C18diacid
  SITE (3)..(8): /note"Disulphide bridge between Cys residues"
  MOD_RES (24)..(24): (S)-2-amino-2-methyl-3-phenylpropanoic acid
XKCNTATCATQRLAEFLRHSSNNXGPILPPTNVGSNTY

SEQ ID NO: 13 - protein, 37 aa, Artificial Sequence
  source: /note="Description of Artificial Sequence: Synthetic polypeptide"
  MOD_RES (1)..(1): Lys, wherein the side chain of Lys is connected to gamma-Glu-gamma-Glu-C18diacid
  SITE (2)..(7): /note"Disulphide bridge between Cys residues"
  MOD_RES (23)..(23): (S)-2-amino-2-methyl-3-phenylpropanoic acid
XCNTATCATQRLANFLVHSSNNXGPILPPTNVGSNTY

SEQ ID NO: 14 - protein, 38 aa, Artificial Sequence
  source: /note="Description of Artificial Sequence: Synthetic polypeptide"
  MOD_RES (1)..(1): Lys, wherein the side chain of Lys is connected to gamma-Glu-C18diacid
  SITE (3)..(8): /note"Disulphide bridge between Cys residues"
  MOD_RES (24)..(24): (S)-2-amino-2-methyl-3-phenylpropanoic acid
XKCNTATCATQRLANFLVHSSNNXGPILPPTNVGSNTY

SEQ ID NO: 15 - protein, 38 aa, Artificial Sequence
  source: /note="Description of Artificial Sequence: Synthetic polypeptide"
  MOD_RES (1)..(1): Lys, wherein the side chain of Lys is connected to gamma-Glu-C18diacid
  SITE (3)..(8): /note"Disulphide bridge between Cys residues"
  MOD_RES (24)..(24): (S)-2-amino-2-methyl-3-phenylpropanoic acid
XKCNTATCATQRLANFLRHSSNNXGPILPPTEVGSNTY

SEQ ID NO: 16 - protein, 37 aa, Artificial Sequence
  source: /note="Description of Artificial Sequence: Synthetic polypeptide"
  MOD_RES (1)..(1): Lys, wherein the side chain of Lys is connected to gamma-Glu-C18diacid
  SITE (2)..(7): /note"Disulphide bridge between Cys residues"
  MOD_RES (23)..(23): (S)-2-amino-2-methyl-3-phenylpropanoic acid
XCNTATCATQRLANFLRHSSNNXGPILPPTEVGSNTY

SEQ ID NO: 17 - protein, 37 aa, Artificial Sequence; identical to SEQ ID NO: 16
  source: /note="Description of Artificial Sequence: Synthetic polypeptide"
  MOD_RES (1)..(1): Lys, wherein the side chain of Lys is connected to O2Oc-O2Oc-gamma-Glu-C18diacid
  SITE (2)..(7): /note"Disulphide bridge between Cys residues"
  MOD_RES (23)..(23): (S)-2-amino-2-methyl-3-phenylpropanoic acid

SEQ ID NO: 18 - protein, 37 aa, Artificial Sequence; identical to SEQ ID NO: 16
  source: /note="Description of Artificial Sequence: Synthetic polypeptide"
  MOD_RES (1)..(1): Lys, wherein the side chain of Lys is connected to gamma-Glu-gamma-Glu-C18diacid
  SITE (2)..(7): /note"Disulphide bridge between Cys residues"
  MOD_RES (23)..(23): (S)-2-amino-2-methyl-3-phenylpropanoic acid

SEQ ID NO: 19 - protein, 37 aa, Artificial Sequence
  source: /note="Description of Artificial Sequence: Synthetic polypeptide"
  MOD_RES (1)..(1): Lys, wherein the side chain of Lys is connected to gamma-Glu-C18diacid
  SITE (2)..(7): /note"Disulphide bridge between Cys residues"
  MOD_RES (23)..(23): (S)-2-amino-2-methyl-3-phenylpropanoic acid
XCNTATCATQRLANFLRHSSNNXGPILPPTNVGSNTY

SEQ ID NO: 20 - protein, 37 aa, Artificial Sequence; identical to SEQ ID NO: 19
  source: /note="Description of Artificial Sequence: Synthetic polypeptide"
  MOD_RES (1)..(1): Lys, wherein the side chain of Lys is connected to gamma-Glu-gamma-Glu-C18diacid
  SITE (2)..(7): /note"Disulphide bridge between Cys residues"
  MOD_RES (23)..(23): (S)-2-amino-2-methyl-3-phenylpropanoic acid

SEQ ID NO: 21 - protein, 37 aa, Artificial Sequence
  source: /note="Description of Artificial Sequence: Synthetic polypeptide"
  MOD_RES (1)..(1): Lys, wherein the side chain of Lys is connected to gamma-Glu-gamma-Glu-C18diacid
  SITE (2)..(7): /note"Disulphide bridge between Cys residues"
  MOD_RES (23)..(23): (S)-2-amino-2-methyl-3-phenylpropanoic acid
XCNTATCATQRLANFLVHSSNNXGPILPPTNVGSRTY

SEQ ID NO: 22 - protein, 37 aa, Artificial Sequence
  source: /note="Description of Artificial Sequence: Synthetic polypeptide"
  MOD_RES (1)..(1): Lys, wherein the side chain of Lys is connected to gamma-Glu-gamma-Glu-C18diacid
  SITE (2)..(7): /note"Disulphide bridge between Cys residues"
  MOD_RES (20)..(20): (S)-2-amino-3-hydroxy-2-methylpropanoic acid
XCNTATCATQRLANFLVHSXNNFGPILPPTNVGSNTY

SEQ ID NO: 23 - protein, 37 aa, Artificial Sequence
  source: /note="Description of Artificial Sequence: Synthetic polypeptide"
  MOD_RES (1)..(1): Lys, wherein the side chain of Lys is connected to gamma-Glu-gamma-Glu-C18diacid
  SITE (2)..(7): /note"Disulphide bridge between Cys residues"
  MOD_RES (23)..(23): (S)-2-amino-2-methyl-3-phenylpropanoic acid
XCNTATCATQRLANFLVHSSNNXGPILPPTEVGSNTY

SEQ ID NO: 24 - protein, 37 aa, Artificial Sequence
  source: /note="Description of Artificial Sequence: Synthetic polypeptide"
  MOD_RES (1)..(1): Lys, wherein the side chain of Lys is connected to gamma-Glu-gamma-Glu-C18diacid
  SITE (2)..(7): /note"Disulphide bridge between Cys residues"
  MOD_RES (23)..(23): (S)-2-amino-2-methyl-3-phenylpropanoic acid
XCNTATCATQRLANFLVHSSNNXGPILPPTRVGSNTY

SEQ ID NO: 25 - protein, 37 aa, Artificial Sequence; identical to SEQ ID NO: 24
  source: /note="Description of Artificial Sequence: Synthetic polypeptide"
  MOD_RES (1)..(1): Lys, wherein the side chain of Lys is connected to gamma-Glu-C18diacid
  SITE (2)..(7): /note"Disulphide bridge between Cys residues"
  MOD_RES (23)..(23): (S)-2-amino-2-methyl-3-phenylpropanoic acid

SEQ ID NO: 26 - protein, 37 aa, Artificial Sequence
  source: /note="Description of Artificial Sequence: Synthetic polypeptide"
  MOD_RES (1)..(1): Lys, wherein the side chain of Lys is connected to gamma-Glu-gamma-Glu-C18diacid
  SITE (2)..(7): /note"Disulphide bridge between Cys residues"
  MOD_RES (17)..(17): 2-amino-2-methylpropanoic acid
  MOD_RES (23)..(23): (S)-2-amino-2-methyl-3-phenylpropanoic acid
XCNTATCATQRLANFLXHSSNNXGPILPPTNVGSNTY

SEQ ID NO: 27 - protein, 37 aa, Artificial Sequence
  source: /note="Description of Artificial Sequence: Synthetic polypeptide"
  MOD_RES (1)..(1): Lys, wherein the side chain of Lys is connected to gamma-Glu-gamma-Glu-C18diacid
  SITE (2)..(7): /note"Disulphide bridge between Cys residues"
  MOD_RES (21)..(21): 2,4-diaminobutanoic acid
XCNIATCATQRLANFLVHSSXNFGPILPPTNVGSRTY

SEQ ID NO: 28 - protein, 38 aa, Artificial Sequence
  source: /note="Description of Artificial Sequence: Synthetic polypeptide"
  MOD_RES (1)..(1): Lys, wherein the side chain of Lys is connected to gamma-Glu-C18diacid
  SITE (3)..(8): /note"Disulphide bridge between Cys residues"
  MOD_RES (22)..(22): 2,4-diaminobutanoic acid
XKCNTATCATQRLANFLVHSSXNFGPILPPTEVGSNTY

SEQ ID NO: 29 - protein, 38 aa, Artificial Sequence
  source: /note="Description of Artificial Sequence: Synthetic polypeptide"
  MOD_RES (1)..(1): Lys, wherein the side chain of Lys is connected to gamma-Glu-C18diacid
  SITE (3)..(8): /note"Disulphide bridge between Cys residues"
  MOD_RES (22)..(22): 2,4-diaminobutanoic acid
XKCNTATCATQRLANFLVHSSXNFGPILPPTNVGSNTY

SEQ ID NO: 30 - protein, 38 aa, Artificial Sequence
  source: /note="Description of Artificial Sequence: Synthetic polypeptide"
  MOD_RES (1)..(1): Lys, wherein the side chain of Lys is connected to gamma-Glu-C18diacid
  SITE (3)..(8): /note"Disulphide bridge between Cys residues"
  MOD_RES (18)..(18): 2-amino-2-methylpropanoic acid
  MOD_RES (22)..(22): 2,4-diaminobutanoic acid
XKCNTATCATQRLANFLXHSSXNFGPILPPTEVGSNTY

SEQ ID NO: 31 - protein, 38 aa, Artificial Sequence
  source: /note="Description of Artificial Sequence: Synthetic polypeptide"
  MOD_RES (1)..(1): Lys, wherein the side chain of Lys is connected to gamma-Glu-C18diacid
  SITE (3)..(8): /note"Disulphide bridge between Cys residues"
  MOD_RES (22)..(22): 2,4-diaminobutanoic acid
  MOD_RES (26)..(26): 2-amino-2-methylpropanoic acid
XKCNTATCATQRLANFLVHSSXNFGXILPPTNVGSNTY

SEQ ID NO: 32 - protein, 38 aa, Artificial Sequence
  source: /note="Description of Artificial Sequence: Synthetic polypeptide"
  MOD_RES (1)..(1): Lys, wherein the side chain of Lys is connected to gamma-Glu-C18diacid
  SITE (3)..(8): /note"Disulphide bridge between Cys residues"
  MOD_RES (15)..(15): 2,4-diaminobutanoic acid
  MOD_RES (24)..(24): (S)-2-amino-2-methyl-3-phenylpropanoic acid
XKCNTATCATQRLAXFLVHSSNNXGPILPPTEVGSNTY

SEQ ID NO: 33 - protein, 38 aa, Artificial Sequence
  source: /note="Description of Artificial Sequence: Synthetic polypeptide"
  MOD_RES (1)..(1): Lys, wherein the side chain of Lys is connected to gamma-Glu-C18diacid
  SITE (3)..(8): /note"Disulphide bridge between Cys residues"
  MOD_RES (15)..(15): 2,4-diaminobutanoic acid
XKCNTATCATQRLAXFLVHSSNNFGPILPPTNVGSNTY

SEQ ID NO: 34 - protein, 38 aa, Artificial Sequence
  source: /note="Description of Artificial Sequence: Synthetic polypeptide"
  MOD_RES (1)..(1): Lys, wherein the side chain of Lys is connected to gamma-Glu-C18diacid
  SITE (3)..(8): /note"Disulphide bridge between Cys residues"
  MOD_RES (15)..(15): 2,4-diaminobutanoic acid
XKCNTATCATQRLAXFLVHSSNNFGPILPPTEVGSNTY

SEQ ID NO: 35 - protein, 38 aa, Artificial Sequence; identical to SEQ ID NO: 29
  source: /note="Description of Artificial Sequence: Synthetic polypeptide"
  MOD_RES (1)..(1): Lys, wherein the side chain of Lys is connected to gamma-Glu-C18diacid
  SITE (3)..(8): /note"Disulphide bridge between Cys residues"
  MOD_RES (22)..(22): 2-amino-2-methylpropanoic acid

SEQ ID NO: 36 - protein, 38 aa, Artificial Sequence
  source: /note="Description of Artificial Sequence: Synthetic polypeptide"
  MOD_RES (1)..(1): Lys, wherein the side chain of Lys is connected to gamma-Glu-C18diacid
  SITE (3)..(8): /note"Disulphide bridge between Cys residues"
  MOD_RES (18)..(18): 2-amino-2-methylpropanoic acid
  MOD_RES (22)..(22): 2-amino-2-methylpropanoic acid
XKCNTATCATQRLANFLXHSSXNFGPILPPTNVGSNTY

SEQ ID NO: 37 - protein, 38 aa, Artificial Sequence
  source: /note="Description of Artificial Sequence: Synthetic polypeptide"
  MOD_RES (1)..(1): Lys, wherein the side chain of Lys is connected to gamma-Glu-C18diacid
  SITE (3)..(8): /note"Disulphide bridge between Cys residues"
  MOD_RES (22)..(22): 2-amino-2-methylpropanoic acid
XKCNTATCATQRLANFLSHSSXNFGPILPPTNVGSNTY

SEQ ID NO: 38 - protein, 38 aa, Artificial Sequence
  source: /note="Description of Artificial Sequence: Synthetic polypeptide"
  MOD_RES (1)..(1): Lys, wherein the side chain of Lys is connected to gamma-Glu-C18diacid
  SITE (3)..(8): /note"Disulphide bridge between Cys residues"
  MOD_RES (22)..(22): 2-amino-2-methylpropanoic acid
XKCNTATCATQRLAEFLVHSSXNFGPILPPTNVGSNTY

SEQ ID NO: 39 - protein, 38 aa, Artificial Sequence
  source: /note="Description of Artificial Sequence: Synthetic polypeptide"
  MOD_RES (1)..(1): Lys, wherein the side chain of Lys is connected to gamma-Glu-C18diacid
  SITE (3)..(8): /note"Disulphide bridge between Cys residues"
  MOD_RES (22)..(22): 2-amino-2-methylpropanoic acid
XKCNTATCATQRLANFLEHSSXNFGPILPPTNVGSNTY

SEQ ID NO: 40 - protein, 38 aa, Artificial Sequence
  source: /note="Description of Artificial Sequence: Synthetic polypeptide"
  MOD_RES (1)..(1): Lys, wherein the side chain of Lys is connected to gamma-Glu-C18diacid
  SITE (3)..(8): /note"Disulphide bridge between Cys residues"
  MOD_RES (22)..(22): 2-amino-2-methylpropanoic acid
XKCNTATCATQRLANFLVHSSXNFGPILPPTHVGSNTY

SEQ ID NO: 41 - protein, 38 aa, Artificial Sequence; identical to SEQ ID NO: 28
  source: /note="Description of Artificial Sequence: Synthetic polypeptide"
  MOD_RES (1)..(1): Lys, wherein the side chain of Lys is connected to gamma-Glu-C18diacid
  SITE (3)..(8): /note"Disulphide bridge between Cys residues"
  MOD_RES (22)..(22): 2-amino-2-methylpropanoic acid

SEQ ID NO: 42 - protein, 38 aa, Artificial Sequence
  source: /note="Description of Artificial Sequence: Synthetic polypeptide"
  MOD_RES (1)..(1): Lys, wherein the side chain of Lys is connected to gamma-Glu-C18diacid
  SITE (3)..(8): /note"Disulphide bridge between Cys residues"
  MOD_RES (22)..(22): 2-amino-2-methylpropanoic acid
XKCNTATCATQRLANFLVHSSXNFGPILPPTNVGSETY

SEQ ID NO: 43 - protein, 38 aa, Artificial Sequence
  source: /note="Description of Artificial Sequence: Synthetic polypeptide"
  MOD_RES (1)..(1): Lys, wherein the side chain of Lys is connected to gamma-Glu-C18diacid
  SITE (3)..(8): /note"Disulphide bridge between Cys residues"
  MOD_RES (22)..(22): 2-amino-2-methylpropanoic acid
XKCNTATCATQRLANFLRHSSXNFGPILPPTEVGSNTY

SEQ ID NO: 44 - protein, 37 aa, Artificial Sequence
  source: /note="Description of Artificial Sequence: Synthetic polypeptide"
  MOD_RES (1)..(1): Lys, wherein the side chain of Lys is connected to gamma-Glu-C18diacid
  SITE (2)..(7): /note"Disulphide bridge between Cys residues"
  MOD_RES (21)..(21): 2-amino-2-methylpropanoic acid
XCNTATCATQRLANFLRHSSXNFGPILPPTEVGSNTY

SEQ ID NO: 45 - protein, 37 aa, Artificial Sequence; identical to SEQ ID NO: 44
  source: /note="Description of Artificial Sequence: Synthetic polypeptide"
  MOD_RES (1)..(1): Lys, wherein the side chain of Lys is connected to O2Oc-O2Oc-gamma-Glu-C18diacid
  SITE (2)..(7): /note"Disulphide bridge between Cys residues"
  MOD_RES (21)..(21): 2-amino-2-methylpropanoic acid

SEQ ID NO: 46 - protein, 38 aa, Artificial Sequence
  source: /note="Description of Artificial Sequence: Synthetic polypeptide"
  MOD_RES (1)..(1): Lys, wherein the side chain of Lys is connected to gamma-Glu-C18diacid
  SITE (3)..(8): /note"Disulphide bridge between Cys residues"
  MOD_RES (22)..(22): 2-amino-2-methylpropanoic acid
XKCNTATCATQRLAHFLVHSSXNFGPILPPTNVGSNTY

SEQ ID NO: 47 - protein, 38 aa, Artificial Sequence
  source: /note="Description of Artificial Sequence: Synthetic polypeptide"
  MOD_RES (1)..(1): Lys, wherein the side chain of Lys is connected to gamma-Glu-C18diacid
  SITE (3)..(8): /note"Disulphide bridge between Cys residues"
  MOD_RES (22)..(22): 2-amino-2-methylpropanoic acid
XKCNTATCATQRLAHFLVHSSXNFGPILPPTNVGSETY

SEQ ID NO: 48 - protein, 37 aa, Artificial Sequence
  source: /note="Description of Artificial Sequence: Synthetic polypeptide"
  MOD_RES (1)..(1): Lys, wherein the side chain of Lys is connected to gamma-Glu-C18diacid
  SITE (2)..(7): /note"Disulphide bridge between Cys residues"
  MOD_RES (21)..(21): 2-amino-2-methylpropanoic acid
XCNTATCATQRLANFLRHSSXNFGPILPPTNVGSNTY

SEQ ID NO: 49 - protein, 37 aa, Artificial Sequence
  source: /note="Description of Artificial Sequence: Synthetic polypeptide"
  MOD_RES (1)..(1): Lys, wherein the side chain of Lys is connected to gamma-Glu-gamma-Glu-C18diacid
  SITE (2)..(7): /note"Disulphide bridge between Cys residues"
  MOD_RES (21)..(21): 2-amino-2-methylpropanoic acid
XCNTATCATQRLANFLVHSSXNFGPILPPTEVGSNTY

SEQ ID NO: 50 - protein, 37 aa, Artificial Sequence; identical to SEQ ID NO: 44
  source: /note="Description of Artificial Sequence: Synthetic polypeptide"
  MOD_RES (1)..(1): Lys, wherein the side chain of Lys is connected to gamma-Glu-gamma-Glu-C18diacid
  SITE (2)..(7): /note"Disulphide bridge between Cys residues"
  MOD_RES (21)..(21): 2-amino-2-methylpropanoic acid

SEQ ID NO: 51 - protein, 38 aa, Artificial Sequence
  source: /note="Description of Artificial Sequence: Synthetic polypeptide"
  MOD_RES (1)..(1): Lys, wherein the side chain of Lys is connected to gamma-Glu-C18diacid
  SITE (3)..(8): /note"Disulphide bridge between Cys residues"
  MOD_RES (22)..(22): 2-amino-2-methylpropanoic acid
XKCNTATCATQRLANFLSHSSXNFGPILPPTHVGSNTY

SEQ ID NO: 52 - protein, 38 aa, Artificial Sequence
  source: /note="Description of Artificial Sequence: Synthetic polypeptide"
  MOD_RES (1)..(1): Lys, wherein the side chain of Lys is connected to gamma-Glu-C18diacid
  SITE (3)..(8): /note"Disulphide bridge between Cys residues"
  MOD_RES (22)..(22): 2-amino-2-methylpropanoic acid
XKCNTATCATQRLANFLSHSSXNFGPILPPTRVGSNTY

SEQ ID NO: 53 - protein, 38 aa, Artificial Sequence
  source: /note="Description of Artificial Sequence: Synthetic polypeptide"
  MOD_RES (1)..(1): Lys, wherein the side chain of Lys is connected to gamma-Glu-C18diacid
  SITE (3)..(8): /note"Disulphide bridge between Cys residues"
  MOD_RES (22)..(22): 2-amino-2-methylpropanoic acid
XKCNTATCATQRLANFLSHSSXNFGPILPPTPVGSNTY

SEQ ID NO: 54 - protein, 38 aa, Artificial Sequence
  source: /note="Description of Artificial Sequence: Synthetic polypeptide"
  MOD_RES (1)..(1): Lys, wherein the side chain of Lys is connected to gamma-Glu-C18diacid
  SITE (3)..(8): /note"Disulphide bridge between Cys residues"
  MOD_RES (22)..(22): 2-amino-2-methylpropanoic acid
XKCNTATCATQRLANFLSHSSXNFGPILPPTNVPSNTY

SEQ ID NO: 55 - protein, 38 aa, Artificial Sequence
  source: /note="Description of Artificial Sequence: Synthetic polypeptide"
  MOD_RES (1)..(1): Lys, wherein the side chain of Lys is connected to gamma-Glu-C18diacid
  SITE (3)..(8): /note"Disulphide bridge between Cys residues"
  MOD_RES (22)..(22): 2-amino-2-methylpropanoic acid
XKCNTATCATQRLANFLSHSSXNFGPILPPTNVGSPTY

SEQ ID NO: 56 - protein, 37 aa, Artificial Sequence
  source: /note="Description of Artificial Sequence: Synthetic polypeptide"
  MOD_RES (1)..(1): Lys, wherein the side chain of Lys is connected to gamma-Glu-C18diacid
  SITE (2)..(7): /note"Disulphide bridge between Cys residues"
  MOD_RES (21)..(21): 2-amino-2-methylpropanoic acid
XCNTATCATQRLANFLVHSSXNFGPILPPTNVGSNTY

SEQ ID NO: 57 - protein, 38 aa, Artificial Sequence; identical to SEQ ID NO: 29
  source: /note="Description of Artificial Sequence: Synthetic polypeptide"
  MOD_RES (1)..(1): Lys, wherein the side chain of Lys is connected to gamma-Glu-gamma-Glu-C18diacid
  SITE (3)..(8): /note"Disulphide bridge between Cys residues"
  MOD_RES (22)..(22): 2-amino-2-methylpropanoic acid

SEQ ID NO: 58 - protein, 38 aa, Artificial Sequence
  source: /note="Description of Artificial Sequence: Synthetic polypeptide"
  MOD_RES (1)..(1): Lys, wherein the side chain of Lys is connected to gamma-Glu-C18diacid
  SITE (3)..(8): /note"Disulphide bridge between Cys residues"
  MOD_RES (22)..(22): 2-amino-2-methylpropanoic acid
XKCNTATCATQRLANFLVHSSXNFGPILPPTNVGSNTP

SEQ ID NO: 59 - protein, 37 aa, Artificial Sequence
  source: /note="Description of Artificial Sequence: Synthetic polypeptide"
  MOD_RES (1)..(1): Lys, wherein the side chain of Lys is connected to gamma-Glu-C18diacid
  SITE (2)..(7): /note"Disulphide bridge between Cys residues"
  MOD_RES (21)..(21): 2-amino-2-methylpropanoic acid
  MOD_RES (27)..(27): D-Leu
XCNTATCATQRLANFLVHSSXNFGPIXPPTNVGSNTY

SEQ ID NO: 60 - protein, 37 aa, Artificial Sequence
  source: /note="Description of Artificial Sequence: Synthetic polypeptide"
  MOD_RES (1)..(1): Lys, wherein the side chain of Lys is connected to gamma-Glu-C18diacid
  SITE (2)..(7): /note"Disulphide bridge between Cys residues"
  MOD_RES (21)..(21): 2-amino-2-methylpropanoic acid
  MOD_RES (28)..(28): D-Pro
XCNTATCATQRLANFLVHSSXNFGPILXPTNVGSNTY

SEQ ID NO: 61 - protein, 37 aa, Artificial Sequence
  source: /note="Description of Artificial Sequence: Synthetic polypeptide"
  MOD_RES (1)..(1): Lys, wherein the side chain of Lys is connected to gamma-Glu-C18diacid
  SITE (2)..(7): /note"Disulphide bridge between Cys residues"
  MOD_RES (21)..(21): 2-amino-2-methylpropanoic acid
  MOD_RES (26)..(26): D-Ile
XCNTATCATQRLANFLVHSSXNFGPXLPPTNVGSNTY

SEQ ID NO: 62 - protein, 37 aa, Artificial Sequence
  source: /note="Description of Artificial Sequence: Synthetic polypeptide"
  MOD_RES (1)..(1): Lys, wherein the side chain of Lys is connected to gamma-Glu-C18diacid
  SITE (2)..(7): /note"Disulphide bridge between Cys residues"
  MOD_RES (16)..(16): D-Leu
  MOD_RES (21)..(21): 2-amino-2-methylpropanoic acid
XCNTATCATQRLANFXVHSSXNFGPILPPTNVGSNTY

SEQ ID NO: 63 - protein, 37 aa, Artificial Sequence
  source: /note="Description of Artificial Sequence: Synthetic polypeptide"
  MOD_RES (1)..(1): Lys, wherein the side chain of Lys is connected to gamma-Glu-C18diacid
  SITE (2)..(7): /note"Disulphide bridge between Cys residues"
  MOD_RES (21)..(21): 2-amino-2-methylpropanoic acid
XCNTATCATQRLANFLVHSSXNFGPILPPTRVGSNTY

SEQ ID NO: 64 - protein, 37 aa, Artificial Sequence
  source: /note="Description of Artificial Sequence: Synthetic polypeptide"
  MOD_RES (1)..(1): Lys, wherein the side chain of Lys is connected to gamma-Glu-C18diacid
  SITE (2)..(7): /note"Disulphide bridge between Cys residues"
  MOD_RES (21)..(21): 2-amino-2-methylpropanoic acid
XCNTATCATQRLANFLVHSSXNFGPILPPTNVGSRTY

SEQ ID NO: 65 - protein, 38 aa, Artificial Sequence
  source: /note="Description of Artificial Sequence: Synthetic polypeptide"
  MOD_RES (1)..(1): Lys, wherein the side chain of Lys is connected to gamma-Glu-C18diacid
  SITE (3)..(8): /note"Disulphide bridge between Cys residues"
  MOD_RES (22)..(22): 2-amino-2-methylpropanoic acid
XKCNTATCATQRLANFLRHSSXNFGPILPPTNVGSNTY

SEQ ID NO: 66 - protein, 38 aa, Artificial Sequence; identical to SEQ ID NO: 65
  source: /note="Description of Artificial Sequence: Synthetic polypeptide"
  MOD_RES (1)..(1): Lys, wherein the side chain of Lys is connected to gamma-Glu-gamma-Glu-C18diacid
  SITE (3)..(8): /note"Disulphide bridge between Cys residues"
  MOD_RES (22)..(22): 2-amino-2-methylpropanoic acid

SEQ ID NO: 67 - protein, 37 aa, Artificial Sequence; identical to SEQ ID NO: 63
  source: /note="Description of Artificial Sequence: Synthetic polypeptide"
  MOD_RES (1)..(1): Lys, wherein the side chain of Lys is connected to gamma-Glu-gamma-Glu-C18diacid
  SITE (2)..(7): /note"Disulphide bridge between Cys residues"
  MOD_RES (21)..(21): 2-amino-2-methylpropanoic acid

SEQ ID NO: 68 - protein, 37 aa, Artificial Sequence; identical to SEQ ID NO: 63
  source: /note="Description of Artificial Sequence: Synthetic polypeptide"
  MOD_RES (1)..(1): C18diacid-gamma-Glu
  SITE (2)..(7): /note"Disulphide bridge between Cys residues"
  MOD_RES (21)..(21): 2-amino-2-methylpropanoic acid

SEQ ID NO: 69 - protein, 38 aa, Artificial Sequence
  source: /note="Description of Artificial Sequence: Synthetic polypeptide"
  MOD_RES (1)..(1): Lys, wherein the side chain of Lys is connected to gamma-Glu-C18diacid
  SITE (3)..(8): /note"Disulphide bridge between Cys residues"
  MOD_RES (22)..(22): 2-amino-2-methylpropanoic acid
XKCNTATCATQRLANFLVHSSXNFGPILPPTRVGSNTY

SEQ ID NO: 70 - protein, 38 aa, Artificial Sequence; identical to SEQ ID NO: 69
  source: /note="Description of Artificial Sequence: Synthetic polypeptide"
  MOD_RES (1)..(1): Lys, wherein the side chain of Lys is connected to gamma-Glu-gamma-Glu-C18diacid
  SITE (3)..(8): /note"Disulphide bridge between Cys residues"
  MOD_RES (22)..(22): 2-amino-2-methylpropanoic acid

SEQ ID NO: 71 - protein, 38 aa, Artificial Sequence; identical to SEQ ID NO: 69
  source: /note="Description of Artificial Sequence: Synthetic polypeptide"
  MOD_RES (1)..(1): C18diacid-gamma-Glu
  SITE (3)..(8): /note"Disulphide bridge between Cys residues"
  MOD_RES (22)..(22): 2-amino-2-methylpropanoic acid

SEQ ID NO: 72 - protein, 37 aa, Artificial Sequence; identical to SEQ ID NO: 64
  source: /note="Description of Artificial Sequence: Synthetic polypeptide"
  MOD_RES (1)..(1): Lys, wherein the side chain of Lys is connected to gamma-Glu-gamma-Glu-C18diacid
  SITE (2)..(7): /note"Disulphide bridge between Cys residues"
  MOD_RES (21)..(21): 2-amino-2-methylpropanoic acid

SEQ ID NO: 73 - protein, 38 aa, Artificial Sequence
  source: /note="Description of Artificial Sequence: Synthetic polypeptide"
  MOD_RES (1)..(1): Lys, wherein the side chain of Lys is connected to gamma-Glu-C18diacid
  SITE (3)..(8): /note"Disulphide bridge between Cys residues"
  MOD_RES (22)..(22): 2-amino-2-methylpropanoic acid
XKCNTATCATQRLANFLVHSSXNFGPILPPTNVGSRTY

SEQ ID NO: 74 - protein, 38 aa, Artificial Sequence; identical to SEQ ID NO: 73
  source: /note="Description of Artificial Sequence: Synthetic polypeptide"
  MOD_RES (1)..(1): Lys, wherein the side chain of Lys is connected to gamma-Glu-gamma-Glu-C18diacid
  SITE (3)..(8): /note"Disulphide bridge between Cys residues"
  MOD_RES (22)..(22): 2-amino-2-methylpropanoic acid

SEQ ID NO: 75 - protein, 37 aa, Artificial Sequence; identical to SEQ ID NO: 48
  source: /note="Description of Artificial Sequence: Synthetic polypeptide"
  MOD_RES (1)..(1): Lys, wherein the side chain of Lys is connected to gamma-Glu-gamma-Glu-C18diacid
  SITE (2)..(7): /note"Disulphide bridge between Cys residues"
  MOD_RES (21)..(21): 2-amino-2-methylpropanoic acid

SEQ ID NO: 76 - protein, 37 aa, Artificial Sequence
  source: /note="Description of Artificial Sequence: Synthetic polypeptide"
  MOD_RES (1)..(1): Lys, wherein the side chain of Lys is connected to gamma-Glu-C18diacid
  SITE (2)..(7): /note"Disulphide bridge between Cys residues"
  MOD_RES (21)..(21): 2-amino-2-methylpropanoic acid
XCNTATCATQRLANFLRHSSXNFGPILPPTRVGSNTY

SEQ ID NO: 77 - protein, 37 aa, Artificial Sequence; identical to SEQ ID NO: 76
  source: /note="Description of Artificial Sequence: Synthetic polypeptide"
  MOD_RES (1)..(1): Lys, wherein the side chain of Lys is connected to gamma-Glu-gamma-Glu-C18diacid
  SITE (2)..(7): /note"Disulphide bridge between Cys residues"
  MOD_RES (21)..(21): 2-amino-2-methylpropanoic acid

SEQ ID NO: 78 - protein, 38 aa, Artificial Sequence
  source: /note="Description of Artificial Sequence: Synthetic polypeptide"
  MOD_RES (1)..(1): Lys, wherein the side chain of Lys is connected to gamma-Glu-C18diacid
  SITE (3)..(8): /note"Disulphide bridge between Cys residues"
  MOD_RES (22)..(22): 2-amino-2-methylpropanoic acid
  MOD_RES (27)..(27): 2-amino-2-methylpropanoic acid
XKCNTATCATQRLANFLVHSSXNFGPXLPPTNVGSNTY

SEQ ID NO: 79 - protein, 38 aa, Artificial Sequence
  source: /note="Description of Artificial Sequence: Synthetic polypeptide"
  MOD_RES (1)..(1): Lys, wherein the side chain of Lys is connected to gamma-Glu-C18diacid
  SITE (3)..(8): /note"Disulphide bridge between Cys residues"
  MOD_RES (22)..(22): 2-amino-2-methylpropanoic acid
  MOD_RES (28)..(28): 2-amino-2-methylpropanoic acid
XKCNTATCATQRLANFLVHSSXNFGPIXPPTNVGSNTY

SEQ ID NO: 80 - protein, 38 aa, Artificial Sequence
  source: /note="Description of Artificial Sequence: Synthetic polypeptide"
  MOD_RES (1)..(1): Lys, wherein the side chain of Lys is connected to gamma-Glu-C18diacid
  SITE (3)..(8): /note"Disulphide bridge between Cys residues"
  MOD_RES (22)..(22): 2-amino-2-methylpropanoic acid
  MOD_RES (32)..(32): 2-amino-2-methylpropanoic acid
XKCNTATCATQRLANFLVHSSXNFGPILPPTXVGSNTY

SEQ ID NO: 81 - protein, 38 aa, Artificial Sequence
  source: /note="Description of Artificial Sequence: Synthetic polypeptide"
  MOD_RES (1)..(1): Lys, wherein the side chain of Lys is connected to gamma-Glu-C18diacid
  SITE (3)..(8): /note"Disulphide bridge between Cys residues"
  MOD_RES (22)..(22): 2-amino-2-methylpropanoic acid
  MOD_RES (34)..(34): 2-amino-2-methylpropanoic acid
XKCNTATCATQRLANFLVHSSXNFGPILPPTNVXSNTY

SEQ ID NO: 82 - protein, 38 aa, Artificial Sequence
  source: /note="Description of Artificial Sequence: Synthetic polypeptide"
  MOD_RES (1)..(1): Lys, wherein the side chain of Lys is connected to gamma-Glu-C18diacid
  SITE (3)..(8): /note"Disulphide bridge between Cys residues"
  MOD_RES (22)..(22): 2-amino-2-methylpropanoic acid
  MOD_RES (36)..(36): 2-amino-2-methylpropanoic acid
XKCNTATCATQRLANFLVHSSXNFGPILPPTNVGSXTY

SEQ ID NO: 83 - protein, 38 aa, Artificial Sequence
  source: /note="Description of Artificial Sequence: Synthetic polypeptide"
  MOD_RES (1)..(1): Lys, wherein the side chain of Lys is connected to gamma-Glu-C18diacid
  SITE (3)..(8): /note"Disulphide bridge between Cys residues"
  MOD_RES (22)..(22): 2-amino-2-methylpropanoic acid
  MOD_RES (37)..(37): 2-amino-2-methylpropanoic acid
XKCNTATCATQRLANFLVHSSXNFGPILPPTNVGSNXY

SEQ ID NO: 84 - protein, 38 aa, Artificial Sequence
  source: /note="Description of Artificial Sequence: Synthetic polypeptide"
  MOD_RES (1)..(1): Lys, wherein the side chain of Lys is connected to gamma-Glu-C18diacid
  SITE (3)..(8): /note"Disulphide bridge between Cys residues"
  MOD_RES (22)..(22): 2-amino-2-methylpropanoic acid
  MOD_RES (35)..(35): 2-amino-2-methylpropanoic acid
XKCNTATCATQRLANFLVHSSXNFGPILPPTNVGXNTY

SEQ ID NO: 85 - protein, 38 aa, Artificial Sequence
  source: /note="Description of Artificial Sequence: Synthetic polypeptide"
  MOD_RES (1)..(1): Lys, wherein the side chain of Lys is connected to gamma-Glu-C18diacid
  SITE (3)..(8): /note"Disulphide bridge between Cys residues"
  MOD_RES (22)..(22): 2-amino-2-methylpropanoic acid
  MOD_RES (38)..(38): 2-amino-2-methylpropanoic acid
XKCNTATCATQRLANFLVHSSXNFGPILPPTNVGSNTX

SEQ ID NO: 86 - protein, 38 aa, Artificial Sequence
  source: /note="Description of Artificial Sequence: Synthetic polypeptide"
  MOD_RES (1)..(1): Lys, wherein the side chain of Lys is connected to gamma-Glu-C18diacid
  SITE (3)..(8): /note"Disulphide bridge between Cys residues"
  MOD_RES (18)..(18): 2-amino-2-methylpropanoic acid
  MOD_RES (22)..(22): 2-amino-2-methylpropanoic acid
XKCNTATCATQRLAHFLXHSSXNFGPILPPTEVGSNTY

SEQ ID NO: 87 - protein, 38 aa, Artificial Sequence
  source: /note="Description of Artificial Sequence: Synthetic polypeptide"
  MOD_RES (1)..(1): Lys, wherein the side chain of Lys is connected to gamma-Glu-C18diacid
  SITE (3)..(8): /note"Disulphide bridge between Cys residues"
  MOD_RES (18)..(18): 2-amino-2-methylpropanoic acid
  MOD_RES (22)..(22): 2-amino-2-methylpropanoic acid
XKCNTATCATQRLANFLXHSSXNFGPILPPTNVGSNTP

SEQ ID NO: 88 - protein, 38 aa, Artificial Sequence
  source: /note="Description of Artificial Sequence: Synthetic polypeptide"
  MOD_RES (1)..(1): Lys, wherein the side chain of Lys is connected to gamma-Glu-C18diacid
  SITE (3)..(8): /note"Disulphide bridge between Cys residues"
  MOD_RES (22)..(22): 2-amino-2-methylpropanoic acid
  MOD_RES (29)..(29): 2-amino-2-methylpropanoic acid
XKCNTATCATQRLANFLVHSSXNFGPILXPTNVGSNTY

SEQ ID NO: 89 - protein, 37 aa, Artificial Sequence
  source: /note="Description of Artificial Sequence: Synthetic polypeptide"
  MOD_RES (1)..(1): Lys, wherein the side chain of Lys is connected to gamma-Glu-gamma-Glu-C18diacid
  SITE (2)..(7): /note"Disulphide bridge between Cys residues"
  MOD_RES (21)..(21): 2-amino-2-methylpropanoic acid
  MOD_RES (31)..(31): 2-amino-2-methylpropanoic acid
XCNTATCATQRLANFLVHSSXNFGPILPPTXVGSNTY

SEQ ID NO: 90 - protein, 37 aa, Artificial Sequence
  source: /note="Description of Artificial Sequence: Synthetic polypeptide"
  MOD_RES (1)..(1): Lys, wherein the side chain of Lys is connected to gamma-Glu-gamma-Glu-C18diacid
  SITE (2)..(7): /note"Disulphide bridge between Cys residues"
  MOD_RES (21)..(21): 2-amino-2-methylpropanoic acid
  MOD_RES (31)..(31): 2-amino-2-methylpropanoic acid
XCNTATCATQRLANFLRHSSXNFGPILPPTXVGSNTY

SEQ ID NO: 91 - protein, 37 aa, Artificial Sequence
  source: /note="Description of Artificial Sequence: Synthetic polypeptide"
  MOD_RES (1)..(1): Lys, wherein the side chain of Lys is connected to gamma-Glu-gamma-Glu-C18diacid
  SITE (2)..(7): /note"Disulphide bridge between Cys residues"
  MOD_RES (21)..(21): 2-amino-2-methylpropanoic acid
  MOD_RES (35)..(35): 2-amino-2-methylpropanoic acid
XCNTATCATQRLANFLVHSSXNFGPILPPTNVGSXTY

SEQ ID NO: 92 - protein, 37 aa, Artificial Sequence
  source: /note="Description of Artificial Sequence: Synthetic polypeptide"
  MOD_RES (1)..(1): Lys, wherein the side chain of Lys is connected to gamma-Glu-gamma-Glu-C18diacid
  SITE (2)..(7): /note"Disulphide bridge between Cys residues"
  MOD_RES (21)..(21): 2-amino-2-methylpropanoic acid
  MOD_RES (35)..(35): 2-amino-2-methylpropanoic acid
XCNTATCATQRLANFLRHSSXNFGPILPPTNVGSXTY

SEQ ID NO: 93 - protein, 38 aa, Artificial Sequence
  source: /note="Description of Artificial Sequence: Synthetic polypeptide"
  MOD_RES (1)..(1): Lys, wherein the side chain of Lys is connected to gamma-Glu-C18diacid
  SITE (3)..(8): /note"Disulphide bridge between Cys residues"
  MOD_RES (18)..(18): 2-amino-2-methylpropanoic acid
  MOD_RES (22)..(22): 2,4-diaminobutanoic acid
  MOD_RES (26)..(26): 2-amino-2-methylpropanoic acid
XKCNTATCATQRLANFLXHSSXNFGXILPPTNVGSNTY

SEQ ID NO: 94 - protein, 38 aa, Artificial Sequence
  source: /note="Description of Artificial Sequence: Synthetic polypeptide"
  MOD_RES (1)..(1): Lys, wherein the side chain of Lys is connected to gamma-Glu-C18diacid
  SITE (3)..(8): /note"Disulphide bridge between Cys residues"
  MOD_RES (18)..(18): 2-amino-2-methylpropanoic acid
  MOD_RES (27)..(27): 2-amino-2-methylpropanoic acid
XKCNTATCATQRLANFLXHSSNNFGPXLPPTNVGSNTY

SEQ ID NO: 95 - protein, 38 aa, Artificial Sequence
  source: /note="Description of Artificial Sequence: Synthetic polypeptide"
  MOD_RES (1)..(1): Lys, wherein the side chain of Lys is connected to gamma-Glu-C18diacid
  SITE (3)..(8): /note"Disulphide bridge between Cys residues"
  MOD_RES (18)..(18): 2-amino-2-methylpropanoic acid
  MOD_RES (28)..(28): 2-amino-2-methylpropanoic acid
XKCNTATCATQRLANFLXHSSNNFGPIXPPTNVGSNTY

SEQ ID NO: 96 - protein, 38 aa, Artificial Sequence
  source: /note="Description of Artificial Sequence: Synthetic polypeptide"
  MOD_RES (1)..(1): Lys, wherein the side chain of Lys is connected to gamma-Glu-C18diacid
  SITE (3)..(8): /note"Disulphide bridge between Cys residues"
  MOD_RES (18)..(18): 2-amino-2-methylpropanoic acid
  MOD_RES (29)..(29): 2-amino-2-methylpropanoic acid
XKCNTATCATQRLANFLXHSSNNFGPILXPTNVGSNTY

SEQ ID NO: 97 - protein, 38 aa, Artificial Sequence
  source: /note="Description of Artificial Sequence: Synthetic polypeptide"
  MOD_RES (1)..(1): Lys, wherein the side chain of Lys is connected to gamma-Glu-C18diacid
  SITE (3)..(8): /note"Disulphide bridge between Cys residues"
  MOD_RES (18)..(18): 2-amino-2-methylpropanoic acid
  MOD_RES (30)..(30): 2-amino-2-methylpropanoic acid
XKCNTATCATQRLANFLXHSSNNFGPILPXTNVGSNTY

SEQ ID NO: 98 - protein, 38 aa, Artificial Sequence
  source: /note="Description of Artificial Sequence: Synthetic polypeptide"
  MOD_RES (1)..(1): Lys, wherein the side chain of Lys is connected to gamma-Glu-C18diacid
  SITE (3)..(8): /note"Disulphide bridge between Cys residues"
  MOD_RES (18)..(18): 2-amino-2-methylpropanoic acid
  MOD_RES (32)..(32): 2-amino-2-methylpropanoic acid
XKCNTATCATQRLANFLXHSSNNFGPILPPTXVGSNTY

SEQ ID NO: 99 - protein, 38 aa, Artificial Sequence
  source: /note="Description of Artificial Sequence: Synthetic polypeptide"
  MOD_RES (1)..(1): Lys, wherein the side chain of Lys is connected to gamma-Glu-C18diacid
  SITE (3)..(8): /note"Disulphide bridge between Cys residues"
  MOD_RES (18)..(18): 2-amino-2-methylpropanoic acid
  MOD_RES (33)..(33): 2-amino-2-methylpropanoic acid
XKCNTATCATQRLANFLXHSSNNFGPILPPTNXGSNTY

SEQ ID NO: 100 - protein, 38 aa, Artificial Sequence
  source: /note="Description of Artificial Sequence: Synthetic polypeptide"
  MOD_RES (1)..(1): Lys, wherein the side chain of Lys is connected to gamma-Glu-C18diacid
  SITE (3)..(8): /note"Disulphide bridge between Cys residues"
  MOD_RES (18)..(18): 2-amino-2-methylpropanoic acid
  MOD_RES (34)..(34): 2-amino-2-methylpropanoic acid
XKCNTATCATQRLANFLXHSSNNFGPILPPTNVXSNTY

SEQ ID NO: 101 - protein, 38 aa, Artificial Sequence
  source: /note="Description of Artificial Sequence: Synthetic polypeptide"
  MOD_RES (1)..(1): Lys, wherein the side chain of Lys is connected to gamma-Glu-C18diacid
  SITE (3)..(8): /note"Disulphide bridge between Cys residues"
  MOD_RES (18)..(18): 2-amino-2-methylpropanoic acid
  MOD_RES (35)..(35): 2-amino-2-methylpropanoic acid
XKCNTATCATQRLANFLXHSSNNFGPILPPTNVGXNTY

SEQ ID NO: 102 - protein, 38 aa, Artificial Sequence
  source: /note="Description of Artificial Sequence: Synthetic polypeptide"
  MOD_RES (1)..(1): Lys, wherein the side chain of Lys is connected to gamma-Glu-C18diacid
  SITE (3)..(8): /note"Disulphide bridge between Cys residues"
  MOD_RES (18)..(18): 2-amino-2-methylpropanoic acid
  MOD_RES (36)..(36): 2-amino-2-methylpropanoic acid
XKCNTATCATQRLANFLXHSSNNFGPILPPTNVGSXTY

SEQ ID NO: 103 - protein, 37 aa, Artificial Sequence
  source: /note="Description of Artificial Sequence: Synthetic polypeptide"
  MOD_RES (1)..(1): Lys, wherein the side chain of Lys is connected to gamma-Glu-C18diacid
  SITE (2)..(7): /note"Disulphide bridge between Cys residues"
  MOD_RES (27)..(27): D-Leu
XCNTATCATQRLANFLVHSSNNFGPIXPPTNVGSNTY

SEQ ID NO: 104 - protein, 37 aa, Artificial Sequence
  source: /note="Description of Artificial Sequence: Synthetic polypeptide"
  MOD_RES (1)..(1): Lys, wherein the side chain of Lys is connected to gamma-Glu-C18diacid
  SITE (2)..(7): /note"Disulphide bridge between Cys residues"
  MOD_RES (28)..(28): D-Pro
XCNTATCATQRLANFLVHSSNNFGPILXPTNVGSNTY

SEQ ID NO: 105 - protein, 38 aa, Artificial Sequence
  source: /note="Description of Artificial Sequence: Synthetic polypeptide"
  MOD_RES (1)..(1): Lys, wherein the side chain of Lys is connected to gamma-Glu-C18diacid
  SITE (3)..(8): /note"Disulphide bridge between Cys residues"
  MOD_RES (22)..(22): 2,4-diaminobutanoic acid
  MOD_RES (26)..(26): 2-amino-2-methylpropanoic acid
XKCNTATCATQRLANFLSHSSXNFGXILPPTNVGSNTY

SEQ ID NO: 106 - protein, 38 aa, Artificial Sequence
  source: /note="Description of Artificial Sequence: Synthetic polypeptide"
  MOD_RES (1)..(1): Lys, wherein the side chain of Lys is connected to gamma-Glu-C18diacid
  SITE (3)..(8): /note"Disulphide bridge between Cys residues"
  MOD_RES (27)..(27): 2-amino-2-methylpropanoic acid
XKCNTATCATQRLANFLVHSSNNFGPXLPPTNVGSNTY

SEQ ID NO: 107 - protein, 38 aa, Artificial Sequence
  source: /note="Description of Artificial Sequence: Synthetic polypeptide"
  MOD_RES (1)..(1): Lys, wherein the side chain of Lys is connected to gamma-Glu-C18diacid
  SITE (3)..(8): /note"Disulphide bridge between Cys residues"
  MOD_RES (27)..(27): 2-amino-2-methylpropanoic acid
XKCNTATCATQRLANFLRHSSNNFGPXLPPTNVGSNTY

SEQ ID NO: 108 - protein, 38 aa, Artificial Sequence
  source: /note="Description of Artificial Sequence: Synthetic polypeptide"
  MOD_RES (1)..(1): Lys, wherein the side chain of Lys is connected to gamma-Glu-C18diacid
  SITE (3)..(8): /note"Disulphide bridge between Cys residues"
  MOD_RES (28)..(28): 2-amino-2-methylpropanoic acid
XKCNTATCATQRLANFLVHSSNNFGPIXPPTNVGSNTY

SEQ ID NO: 109 - protein, 38 aa, Artificial Sequence
  source: /note="Description of Artificial Sequence: Synthetic polypeptide"
  MOD_RES (1)..(1): Lys, wherein the side chain of Lys is connected to gamma-Glu-C18diacid
  SITE (3)..(8): /note"Disulphide bridge between Cys residues"
  MOD_RES (23)..(23): 2-amino-2-methylpropanoic acid
XKCNTATCATQRLANFLVHSSNXFGPILPPTNVGSNTY

SEQ ID NO: 110 - protein, 38 aa, Artificial Sequence
  source: /note="Description of Artificial Sequence: Synthetic polypeptide"
  MOD_RES (1)..(1): Lys, wherein the side chain of Lys is connected to gamma-Glu-C18diacid
  SITE (3)..(8): /note"Disulphide bridge between Cys residues"
  MOD_RES (25)..(25): 2-amino-2-methylpropanoic acid
XKCNTATCATQRLANFLVHSSNNFXPILPPTNVGSNTY

SEQ ID NO: 111 - protein, 38 aa, Artificial Sequence
  source: /note="Description of Artificial Sequence: Synthetic polypeptide"
  MOD_RES (1)..(1): Lys, wherein the side chain of Lys is connected to gamma-Glu-C18diacid
  SITE (3)..(8): /note"Disulphide bridge between Cys residues"
XKCNTATCATQRLANFLVHSSNHFGPILPPTNVGSETY

SEQ ID NO: 112 - protein, 38 aa, Artificial Sequence; identical to SEQ ID NO: 3
  source: /note="Description of Artificial Sequence: Synthetic polypeptide"
  MOD_RES (1)..(1): C20diacid-gamma-Glu
  SITE (3)..(8): /note"Disulphide bridge between Cys residues"

SEQ ID NO: 113 - protein, 38 aa, Artificial Sequence
  source: /note="Description of Artificial Sequence: Synthetic polypeptide"
  MOD_RES (1)..(1): C20diacid-gamma-Glu
  MOD_RES (2)..(2): O2Oc-O2Oc-Lys
  SITE (3)..(8): /note"Disulphide bridge between Cys residues"
XXCNTATCATQRLANFLVHSSNNFGPILPPTNVGSNTY

SEQ ID NO: 114 - protein, 37 aa, Artificial Sequence
  source: /note="Description of Artificial Sequence: Synthetic polypeptide"
  MOD_RES (1)..(1): Lys, wherein the side chain of Lys is connected to gamma-Glu-gamma-Glu-C20diacid
  SITE (2)..(7): /note"Disulphide bridge between Cys residues"
XCNTATCATQRLANFLVHSSNNFGPILPPTNVGSRTY

SEQ ID NO: 115 - protein, 37 aa, Artificial Sequence
  source: /note="Description of Artificial Sequence: Synthetic polypeptide"
  MOD_RES (1)..(1): Lys, wherein the side chain of Lys is connected to gamma-Glu-gamma-Glu-C20diacid
  SITE (2)..(7): /note"Disulphide bridge between Cys residues"
XCNTATCATQRLANFLVHSSPNFPAILSPTNVGSNTY

SEQ ID NO: 116 - protein, 37 aa, Artificial Sequence
  source: /note="Description of Artificial Sequence: Synthetic polypeptide"
  MOD_RES (1)..(1): Lys, wherein the side chain of Lys is connected to gamma-Glu-gamma-Glu-C20diacid
  SITE (2)..(7): /note"Disulphide bridge between Cys residues"
XCNTATCATQRLAEFLRHSSNNFGPILPPTNVGSNTY

SEQ ID NO: 117 - protein, 37 aa, Artificial Sequence; identical to SEQ ID NO: 8
  source: /note="Description of Artificial Sequence: Synthetic polypeptide"
  MOD_RES (1)..(1): Lys, wherein the side chain of Lys is connected to gamma-Glu-gamma-Glu-C20diacid
  SITE (2)..(7): /note"Disulphide bridge between Cys residues"
  MOD_RES (21)..(21): 2-amino-2-methylpropanoic acid

SEQ ID NO: 118 - protein, 37 aa, Artificial Sequence
  source: /note="Description of Artificial Sequence: Synthetic polypeptide"
  MOD_RES (1)..(1): Lys, wherein the side chain of Lys is connected to gamma-Glu-gamma-Glu-C20diacid
  SITE (2)..(7): /note"Disulphide bridge between Cys residues"
XCNIATCATQRLANFLVHSIANFGPILPPTNVGSRTY

SEQ ID NO: 119 - protein, 37 aa, Artificial Sequence
  source: /note="Description of Artificial Sequence: Synthetic polypeptide"
  MOD_RES (1)..(1): Lys, wherein the side chain of Lys is connected to gamma-Glu-gamma-Glu-C20diacid
  SITE (2)..(7): /note"Disulphide bridge between Cys residues"
XCNTATCATQRLANFLVHSPPNFPAILSPTNVGSNTY

SEQ ID NO: 120 - protein, 37 aa, Artificial Sequence
  source: /note="Description of Artificial Sequence: Synthetic polypeptide"
  MOD_RES (1)..(1): Lys, wherein the side chain of Lys is connected to gamma-Glu-gamma-Glu-C20diacid
  SITE (2)..(7): /note"Disulphide bridge between Cys residues"
XCNAATCATQRLANWLVHSSPNFPAILSPTNVGSNTY

SEQ ID NO: 121 - protein, 37 aa, Artificial Sequence
  source: /note="Description of Artificial Sequence: Synthetic polypeptide"
  MOD_RES (1)..(1): Lys, wherein the side chain of Lys is connected to gamma-Glu-gamma-Glu-C20diacid
  SITE (2)..(7): /note"Disulphide bridge between Cys residues"
  MOD_RES (21)..(21): 2-amino-2-methylpropanoic acid
  MOD_RES (24)..(24): (2S,4R)-4-hydroxypyrrolidine-2-carboxylic acid
XCNTATCATQRLANFLVHSSXNFXAILSPTNVGSNTY

SEQ ID NO: 122 - protein, 37 aa, Artificial Sequence
  source: /note="Description of Artificial Sequence: Synthetic polypeptide"
  MOD_RES (1)..(1): Lys, wherein the side chain of Lys is connected to gamma-Glu-gamma-Glu-C18diacid
  SITE (2)..(7): /note"Disulphide bridge between Cys residues"
  MOD_RES (21)..(21): 2-amino-2-methylpropanoic acid
  MOD_RES (31)..(31): 2,4-diaminobutanoic acid
XCNTATCATQRLANFLVHSSXNFPAILSPTXVGSNTY

SEQ ID NO: 123 - protein, 37 aa, Artificial Sequence; identical to SEQ ID NO: 122
  source: /note="Description of Artificial Sequence: Synthetic polypeptide"
  MOD_RES (1)..(1): Lys, wherein the side chain of Lys is connected to gamma-Glu-gamma-Glu-C20diacid
  SITE (2)..(7): /note"Disulphide bridge between Cys residues"
  MOD_RES (21)..(21): 2-amino-2-methylpropanoic acid
  MOD_RES (31)..(31): 2,4-diaminobutanoic acid

SEQ ID NO: 124 - protein, 37 aa, Artificial Sequence
  source: /note="Description of Artificial Sequence: Synthetic polypeptide"
  MOD_RES (1)..(1): Lys, wherein the side chain of Lys is connected to gamma-Glu-gamma-Glu-C18diacid
  SITE (2)..(7): /note"Disulphide bridge between Cys residues"
  MOD_RES (21)..(21): 2-amino-2-methylpropanoic acid
  MOD_RES (35)..(35): 2,4-diaminobutanoic acid
XCNTATCATQRLANFLVHSSXNFPAILSPTNVGSXTY

SEQ ID NO: 125 - protein, 37 aa, Artificial Sequence; identical to SEQ ID NO: 124
  source: /note="Description of Artificial Sequence: Synthetic polypeptide"
  MOD_RES (1)..(1): Lys, wherein the side chain of Lys is connected to gamma-Glu-gamma-Glu-C20diacid
  SITE (2)..(7): /note"Disulphide bridge between Cys residues"
  MOD_RES (21)..(21): 2-amino-2-methylpropanoic acid
  MOD_RES (35)..(35): 2,4-diaminobutanoic acid

SEQ ID NO: 126 - protein, 38 aa, Artificial Sequence; identical to SEQ ID NO: 36
  source: /note="Description of Artificial Sequence: Synthetic polypeptide"
  MOD_RES (1)..(1): Lys, wherein the side chain of Lys is connected to gamma-Glu-C18diacid
  SITE (3)..(8): /note"Disulphide bridge between Cys residues"
  MOD_RES (18)..(18): 2-amino-2-methylpropanoic acid
  MOD_RES (22)..(22): 2,4-diaminobutanoic acid

SEQ ID NO: 127 - protein, 37 aa, Artificial Sequence
  source: /note="Description of Artificial Sequence: Synthetic polypeptide"
  MOD_RES (1)..(1): Lys, wherein the side chain of Lys is connected to gamma-Glu-gamma-Glu-C18diacid
  SITE (2)..(7): /note"Disulphide bridge between Cys residues"
  MOD_RES (17)..(17): 2-amino-2-methylpropanoic acid
XCNTATCATQRLANFLXHSSNNFGPILPPTNVGSNTY

SEQ ID NO: 128 - protein, 38 aa, Artificial Sequence
  source: /note="Description of Artificial Sequence: Synthetic polypeptide"
  MOD_RES (1)..(1): Lys, wherein the side chain of Lys is connected to gamma-Glu-C18diacid
  SITE (3)..(8): /note"Disulphide bridge between Cys residues"
  MOD_RES (18)..(18): 2-amino-2-methylpropanoic acid
XKCNTATCATQRLAEFLXHSSNNFGPILPPTNVGSNTY

SEQ ID NO: 129 - protein, 38 aa, Artificial Sequence
  source: /note="Description of Artificial Sequence: Synthetic polypeptide"
  MOD_RES (1)..(1): Lys, wherein the side chain of Lys is connected to gamma-Glu-C18diacid
  SITE (3)..(8): /note"Disulphide bridge between Cys residues"
  MOD_RES (18)..(18): 2-amino-2-methylpropanoic acid
XKCNTATCATQRLANFLXHSSNNFGPILPPTNVGSNTY

SEQ ID NO: 130 - protein, 38 aa, Artificial Sequence
  source: /note="Description of Artificial Sequence: Synthetic polypeptide"
  MOD_RES (1)..(1): Lys, wherein the side chain of Lys is connected to gamma-Glu-C18diacid
  SITE (3)..(8): /note"Disulphide bridge between Cys residues"
  MOD_RES (18)..(18): 2-amino-2-methylpropanoic acid
XKCNTATCATQRLAEFLXHSSHNFGPILPPTNVGSNTY

SEQ ID NO: 131 - protein, 38 aa, Artificial Sequence
  source: /note="Description of Artificial Sequence: Synthetic polypeptide"
  MOD_RES (1)..(1): Lys, wherein the side chain of Lys is connected to gamma-Glu-C18diacid
  SITE (3)..(8): /note"Disulphide bridge between Cys residues"
  MOD_RES (18)..(18): 2-amino-2-methylpropanoic acid
XKCNTATCATQRLANFLXHSSHNFGPILPPTNVGSNTY

SEQ ID NO: 132 - protein, 38 aa, Artificial Sequence
  source: /note="Description of Artificial Sequence: Synthetic polypeptide"
  MOD_RES (1)..(1): Lys, wherein the side chain of Lys is connected to gamma-Glu-C18diacid
  SITE (3)..(8): /note"Disulphide bridge between Cys residues"
  MOD_RES (18)..(18): 2-amino-2-methylpropanoic acid
XKCNTATCATQRLANFLXHSSPNFGPILPPTNVGSNTY

SEQ ID NO: 133 - protein, 38 aa, Artificial Sequence
  source: /note="Description of Artificial Sequence: Synthetic polypeptide"
  MOD_RES (1)..(1): Lys, wherein the side chain of Lys is connected to gamma-Glu-C18diacid
  SITE (3)..(8): /note"Disulphide bridge between Cys residues"
  MOD_RES (18)..(18): 2-amino-2-methylpropanoic acid
XKCNTATCATQRLANFLXHSSSNFGPILPPTNVGSNTY

SEQ ID NO: 134 - protein, 38 aa, Artificial Sequence
  source: /note="Description of Artificial Sequence: Synthetic polypeptide"
  MOD_RES (1)..(1): Lys, wherein the side chain of Lys is connected to gamma-Glu-C18diacid
  SITE (3)..(8): /note"Disulphide bridge between Cys residues"
  MOD_RES (18)..(18): 2-amino-2-methylpropanoic acid
XKCNTATCATQRLANFLXHSSNNFGPILPPTPVGSNTY

SEQ ID NO: 135 - protein, 38 aa, Artificial Sequence
  source: /note="Description of Artificial Sequence: Synthetic polypeptide"
  MOD_RES (1)..(1): Lys, wherein the side chain of Lys is connected to gamma-Glu-C18diacid
  SITE (3)..(8): /note"Disulphide bridge between Cys residues"
  MOD_RES (18)..(18): 2-amino-2-methylpropanoic acid
XKCNTATCATQRLANFLXHSSNHFGPILPPTNVGSNTY

SEQ ID NO: 136 - protein, 38 aa, Artificial Sequence
  source: /note="Description of Artificial Sequence: Synthetic polypeptide"
  MOD_RES (1)..(1): Lys, wherein the side chain of Lys is connected to gamma-Glu-C18diacid
  SITE (3)..(8): /note"Disulphide bridge between Cys residues"
  MOD_RES (18)..(18): 2-amino-2-methylpropanoic acid
XKCNTATCATQRLANFLXHSSNNFGPILPPTNVGSNTP

SEQ ID NO: 137 - protein, 38 aa, Artificial Sequence
  source: /note="Description of Artificial Sequence: Synthetic polypeptide"
  MOD_RES (1)..(1): Lys, wherein the side chain of Lys is connected to gamma-Glu-C18diacid
  SITE (3)..(8): /note"Disulphide bridge between Cys residues"
  MOD_RES (18)..(18): 2-amino-2-methylpropanoic acid
XKCNTATCATQRLANFLXHSSRNFGPILPPTNVGSNTY

SEQ ID NO: 138 - protein, 38 aa, Artificial Sequence
  source: /note="Description of Artificial Sequence: Synthetic polypeptide"
  MOD_RES (1)..(1): Lys, wherein the side chain of Lys is connected to gamma-Glu-C18diacid
  SITE (3)..(8): /note"Disulphide bridge between Cys residues"
  MOD_RES (18)..(18): 2-amino-2-methylpropanoic acid
XKCNTATCATQRLANFLXHSSPNFGPILPPTEVGSNTY

SEQ ID NO: 139 - protein, 38 aa, Artificial Sequence
  source: /note="Description of Artificial Sequence: Synthetic polypeptide"
  MOD_RES (1)..(1): Lys, wherein the side chain of Lys is connected to gamma-Glu-C18diacid
  SITE (3)..(8): /note"Disulphide bridge between Cys residues"
  MOD_RES (18)..(18): 2-amino-2-methylpropanoic acid
XKCNTATCATQRLANFLXHSSPNFGPILPPTNVGSETY

SEQ ID NO: 140 - protein, 38 aa, Artificial Sequence
  source: /note="Description of Artificial Sequence: Synthetic polypeptide"
  MOD_RES (1)..(1): Lys, wherein the side chain of Lys is connected to gamma-Glu-C18diacid
  SITE (3)..(8): /note"Disulphide bridge between Cys residues"
  MOD_RES (18)..(18): 2-amino-2-methylpropanoic acid
XKCNTATCATQRLANFLXHSSNNFGPILPPTEVGSNTY

SEQ ID NO: 141 - protein, 38 aa, Artificial Sequence
  source: /note="Description of Artificial Sequence: Synthetic polypeptide"
  MOD_RES (1)..(1): Lys, wherein the side chain of Lys is connected to gamma-Glu-C18diacid
  SITE (3)..(8): /note"Disulphide bridge between Cys residues"
  MOD_RES (18)..(18): 2-amino-2-methylpropanoic acid
XKCNTATCATQRLANFLXHSSNNFGPILPPTNVGSRTY

SEQ ID NO: 142 - protein, 38 aa, Artificial Sequence
  source: /note="Description of Artificial Sequence: Synthetic polypeptide"
  MOD_RES (1)..(1): Lys, wherein the side chain of Lys is connected to gamma-Glu-C18diacid
  SITE (3)..(8): /note"Disulphide bridge between Cys residues"
  MOD_RES (18)..(18): 2-amino-2-methylpropanoic acid
XKCNTATCATQRLANFLXHSSNNFGPILPPTNVGSETY

SEQ ID NO: 143 - protein, 40 aa, Artificial Sequence
  source: /note="Description of Artificial Sequence: Synthetic polypeptide"
  MOD_RES (1)..(1): Lys, wherein the side chain of Lys is connected to gamma-Glu-C18diacid
  SITE (5)..(10): /note"Disulphide bridge between Cys residues"
  MOD_RES (20)..(20): 2-amino-2-methylpropanoic acid
XGGKCNTATCATQRLANFLXHSSNNFGPILPPTNVGSNTY

SEQ ID NO: 144 - protein, 37 aa, Artificial Sequence
  source: /note="Description of Artificial Sequence: Synthetic polypeptide"
  MOD_RES (1)..(1): Lys, wherein the side chain of Lys is connected to gamma-Glu-C18diacid
  SITE (2)..(7): /note"Disulphide bridge between Cys residues"
  MOD_RES (17)..(17): 2-amino-2-methylpropanoic acid
XCNTATCATQRLAHFLXHSSNNFGPILPPTNVGSNTY

SEQ ID NO: 145 - protein, 38 aa, Artificial Sequence
  source: /note="Description of Artificial Sequence: Synthetic polypeptide"
  MOD_RES (1)..(1): Lys, wherein the side chain of Lys is connected to gamma-Glu-C18diacid
  SITE (3)..(8): /note"Disulphide bridge between Cys residues"
  MOD_RES (18)..(18): 2-amino-2-methylpropanoic acid
XKCNTATCATQRLANFLXHSSNNFGPILPPTNVGHNTY

SEQ ID NO: 146 - protein, 38 aa, Artificial Sequence
  source: /note="Description of Artificial Sequence: Synthetic polypeptide"
  MOD_RES (1)..(1): Lys, wherein the side chain of Lys is connected to gamma-Glu-C18diacid
  SITE (3)..(8): /note"Disulphide bridge between Cys residues"
  MOD_RES (18)..(18): 2-amino-2-methylpropanoic acid
XKCNTATCATQRLANFLXHSSNNFGPILPPTHVGSETY

SEQ ID NO: 147 - protein, 38 aa, Artificial Sequence
  source: /note="Description of Artificial Sequence: Synthetic polypeptide"
  MOD_RES (1)..(1): Lys, wherein the side chain of Lys is connected to gamma-Glu-C18diacid
  SITE (3)..(8): /note"Disulphide bridge between Cys residues"
  MOD_RES (18)..(18): 2-amino-2-methylpropanoic acid
XKCNTATCATQRLANFLXHSSNHFGPILPPTNVGSETY

SEQ ID NO: 148 - protein, 38 aa, Artificial Sequence
  source: /note="Description of Artificial Sequence: Synthetic polypeptide"
  MOD_RES (1)..(1): Lys, wherein the side chain of Lys is connected to gamma-Glu-C18diacid
  SITE (3)..(8): /note"Disulphide bridge between Cys residues"
  MOD_RES (18)..(18): 2-amino-2-methylpropanoic acid
XKCNTATCATQRLANFLXHSSNNFGPILPPTNVGPNTY

SEQ ID NO: 149 - protein, 37 aa, Artificial Sequence; identical to SEQ ID NO: 127
  source: /note="Description of Artificial Sequence: Synthetic polypeptide"
  MOD_RES (1)..(1): Lys, wherein the side chain of Lys is connected to gamma-Glu-C18diacid
  SITE (2)..(7): /note"Disulphide bridge between Cys residues"
  MOD_RES (17)..(17): 2-amino-2-methylpropanoic acid

SEQ ID NO: 150 - protein, 37 aa, Artificial Sequence
  source: /note="Description of Artificial Sequence: Synthetic polypeptide"
  MOD_RES (1)..(1): Lys, wherein the side chain of Lys is connected to gamma-Glu-C18diacid
  SITE (2)..(7): /note"Disulphide bridge between Cys residues"
  MOD_RES (17)..(17): 2-amino-2-methylpropanoic acid
  MOD_RES (21)..(21): 2,4-diaminobutanoic acid
XCNTATCATQRLANFLXHSSXNFGPILPPTNVGSNTY

SEQ ID NO: 151 - protein, 37 aa, Artificial Sequence
  source: /note="Description of Artificial Sequence: Synthetic polypeptide"
  MOD_RES (1)..(1): Lys, wherein the side chain of Lys is connected to gamma-Glu-C18diacid
  SITE (2)..(7): /note"Disulphide bridge between Cys residues"
  MOD_RES (17)..(17): 2-amino-2-methylpropanoic acid
  MOD_RES (27)..(27): D-Leu
XCNTATCATQRLANFLXHSSNNFGPIXPPTNVGSNTY

SEQ ID NO: 152 - protein, 38 aa, Artificial Sequence
  source: /note="Description of Artificial Sequence: Synthetic polypeptide"
  MOD_RES (1)..(1): Lys, wherein the side chain of Lys is connected to gamma-Glu-C18diacid
  SITE (3)..(8): /note"Disulphide bridge between Cys residues"
  MOD_RES (18)..(18): 2-amino-2-methylpropanoic acid
XKCNTATCATQRLANFLXHSSNNFGPRLPPTNVGSNTY

SEQ ID NO: 153 - protein, 38 aa, Artificial Sequence
  source: /note="Description of Artificial Sequence: Synthetic polypeptide"
  MOD_RES (1)..(1): Lys, wherein the side chain of Lys is connected to gamma-Glu-C18diacid
  SITE (3)..(8): /note"Disulphide bridge between Cys residues"
  MOD_RES (18)..(18): 2-amino-2-methylpropanoic acid
XKCNTATCATQRLANFLXHSSKNFGPILPPTNVGSNTY

SEQ ID NO: 154 - protein, 38 aa, Artificial Sequence
  source: /note="Description of Artificial Sequence: Synthetic polypeptide"
  MOD_RES (1)..(1): Lys, wherein the side chain of Lys is connected to gamma-Glu-C18diacid
  SITE (3)..(8): /note"Disulphide bridge between Cys residues"
  MOD_RES (18)..(18): 2-amino-2-methylpropanoic acid
XKCNTATCATQRLANFLXHSSGNFGPILPPTNVGSNTY

SEQ ID NO: 155 - protein, 37 aa, Artificial Sequence
  source: /note="Description of Artificial Sequence: Synthetic polypeptide"
  MOD_RES (1)..(1): Lys, wherein the side chain of Lys is connected to gamma-Glu-C18diacid
  SITE (2)..(7): /note"Disulphide bridge between Cys residues"
  MOD_RES (17)..(17): 2-amino-2-methylpropanoic acid
XCNTATCATQRLANFLXHSSNNFGPILPPTRVGSNTY

SEQ ID NO: 156 - protein, 38 aa, Artificial Sequence
  source: /note="Description of Artificial Sequence: Synthetic polypeptide"
  MOD_RES (1)..(1): Lys, wherein the side chain of Lys is connected to gamma-Glu-C18diacid
  SITE (3)..(8): /note"Disulphide bridge between Cys residues"
  MOD_RES (15)..(15): 2,4-diaminobutanoic acid
  MOD_RES (18)..(18): 2-amino-2-methylpropanoic acid
XKCNTATCATQRLAXFLXHSSNNFGPILPPTEVGSNTY

SEQ ID NO: 157 - protein, 37 aa, Artificial Sequence; identical to SEQ ID NO: 89
  source: /note="Description of Artificial Sequence: Synthetic polypeptide"
  MOD_RES (1)..(1): Lys, wherein the side chain of Lys is connected to C18diacid
  SITE (2)..(7): /note"Disulphide bridge between Cys residues"
  MOD_RES (21)..(21): 2-amino-2-methylpropanoic acid
  MOD_RES (31)..(31): 2-amino-2-methylpropanoic acid

SEQ ID NO: 158 - protein, 37 aa, Artificial Sequence; identical to SEQ ID NO: 89
  source: /note="Description of Artificial Sequence: Synthetic polypeptide"
  MOD_RES (1)..(1): Lys, wherein the side chain of Lys is connected to C18diacid
  SITE (2)..(7): /note"Disulphide bridge between Cys residues"
  MOD_RES (21)..(21): 2-amino-2-methylpropanoic acid
  MOD_RES (31)..(31): 2-amino-2-methylpropanoic acid

SEQ ID NO: 159 - protein, 41 aa, Artificial Sequence; identical to SEQ ID NO: 2
  source: /note="Description of Artificial Sequence: Synthetic polypeptide"
  MOD_RES (1)..(1): Lys (linker-lipid) or absent
  VARIANT (2)..(2): /replace=" "
  VARIANT (3)..(3): /replace=" "
  VARIANT (4)..(4): /replace="Lys (linker-lipid)" or " "
  VARIANT (5)..(5): /replace="Lys (linker-lipid)"or " "
  VARIANT (8)..(8): /replace="Ile" or "Ala"
  VARIANT (18)..(18): /replace="His" or "Glu" or "2,4-diaminobutanoic acid (Dab)" or "alpha methyl amino acid"
  VARIANT (19)..(19): /replace="Trp"
  VARIANT (20)..(20): /replace="D-Leu"
  VARIANT (21)..(21): /replace="Ser" or "Glu" or "Arg" or "(2S,4R)-4-hydroxypyrrolidine -2-carboxylic acid (Hyp)" or "Dab" or "alpha methyl amino acid"
  VARIANT (24)..(24): /replace="Ile" or "Pro" or "alpha methyl amino acid"
  VARIANT (25)..(25): /replace="Dab" or "His" or "Pro" or "Ser" or "Arg" or "Lys" or "Gly" or "Glu" or "Ala" or "Hyp " or "alpha methyl amino acid"
  VARIANT (26)..(26): /replace="His" or "Hyp" or "Dab" or "alpha methyl amino acid"
  VARIANT (27)..(27): /replace="Hyp" or "alpha methyl amino acid"
  VARIANT (28)..(28): /replace="Pro" or "Hyp" or "alpha methyl amino acid"
  VARIANT (29)..(29): /replace="Ala" or "Hyp" or "alpha methyl amino acid"
  VARIANT (30)..(30): /replace="D-Ile" or "Arg" or "Hyp" or "alpha methyl amino acid"
  VARIANT (31)..(31): /replace="D-Leu" or "Hyp" or "alpha methyl amino acid"
  VARIANT (32)..(32): /replace="D-Pro" or "Ser" or "Hyp" or "alpha methyl amino acid"
  VARIANT (33)..(33): /replace="Hyp" or "alpha methyl amino acid"
  VARIANT (35)..(35): /replace="Glu" or "His" or "Arg" or "Pro" or "Dab" or "alpha methyl amino acid"
  VARIANT (36)..(36): /replace="Hyp" or "Dab" or "alpha methyl amino acid"
  VARIANT (37)..(37): /replace="Pro" or "Hyp" or "alpha methyl amino acid"
  VARIANT (38)..(38): /replace="Pro" or "His" or "Hyp" or "alpha methyl amino acid"
  VARIANT (39)..(39): /replace="Pro" or "Arg" or "Glu" or "Dab" or "Hyp" or "alpha methyl amino acid"
  VARIANT (40)..(40): /replace="Hyp" or "alpha methyl amino acid"
  VARIANT (41)..(41): /replace="Pro" or "Hyp" or "alpha methyl amino acid"
  SITE (1)..(41): /note="Variant residues given in the sequence have no preference with respect to those in the annotations for variant positions"